European Patent Application EP 4 273 251 A1, published November 8, 2023. Title: Recombinant Bacillus genus microorganism and Method for producing human milk oligosaccharides using the same. Applicant: SAMYANG CORPORATION. The sequence listing filed with the application follows.

SEQUENCE LISTING (31 sequences)

SEQ ID NO: 1 - protein, 261 aa, Artificial Sequence
  Amino acid sequence of Am2FT_2
MNMERKTGLMNKKYVSPCFLPGMRLGNIMFTLAAACAHARTVGVECRVPWAYNDASLMLRSRLGGWVLPSTPCGTNEPPSWQEPSFAYCPVPSRIRTGGLRGYFQSARYFEGQEAFIRALFAPLTAEKEPGAVGIHIRLGDYRRLRDKHRILDPGFLRRAAGHLSSGKNRLVLFSDEPDEAAEMLARVPAFGRFALEIDRGAPCESLRRMTAMEELVMSCSSFSWWGAWLGNTRKVIVPRDWFVGGVEDYRDIYLPHWVTL

SEQ ID NO: 2 - protein, 291 aa, Artificial Sequence
  Amino acid sequence of Bm2FT
MKIVQISSGLGNQLFQYALYKRLSMNNNDVFLDVETSYQLNKNQHNGYEIERIFSIQPSHATKGMIDELADVDNRLINRLRRKLFGPKNSMYTETKEFSYDCEVFTKDGIYIKGYWQNYNYFKEIEDDLKNELVFKKALDLKNSHLINQMNKEISVSIHVRRGDYYLNKEYENKFGNIADLDYYLKAINFIKKEVDDPKFYVFSDDIKWAKENLNLTDNVTYVEHNKGSDSYKDMRLMTCCKHNIIANSTFSWWGAFLNENKNKIVIAPGKWINVEGVGGINLFPEGWIVY

SEQ ID NO: 3 - protein, 299 aa, Artificial Sequence
  Amino acid sequence of Bm2FT_2
MGCIKRLFLYEYGGRCFLVIVKIKGGFGNQLFTYASAYAISQELQQNLIMDKVIYDLDYFRKFELPSLSLKYDQMLISKFVPNTKVKTLIYKVLRRLKLKGFTEVHEKKEFSFDENIYNLSGDIYLDGYWQNYRYFHKYYKDLSEMFVPRETPRKEVTDYITSLRGVNSVAMHVRRGDYKTFNGGKCLSLDYYIKAMEYFNSNDVQFYVFTDDIDFCEKNLPNSENINYVSRSEKLTDIEEFFIMKECKNFIIANSSFSWWAAYLSEQKADSLIVAPVVDMWKRDFYPDEWVALNTHLE

SEQ ID NO: 4 - protein, 287 aa, Artificial Sequence
  Amino acid sequence of Bm2FT_3
MIIVQIKGGLGNQLFSYASAYGIARENETELIIDRYIYDTSYSLRKYMLDFFPEIDEALLLKYIPKKNKISQIMYKLIRKSKLKYKYKAQLFLEEEEFKFTRISTQNENLYLNGYWQSYVYFDKYRNDIIKKFTPLVSFNQDGNQLLNEIKSYNSVAIHVRRGDYINFKGGKCLDSSYYIKAMKHLYNLKGKNLFFYIFTDDVEYCKRIFKNVANVKFIGEEAKLSDFEEFTLMTHCKNLIIGNSSFSWWAAYLASCKDKAVIAPVVDMWTEDFYLPEWIKIKADLQ

SEQ ID NO: 5 - protein, 291 aa, Artificial Sequence
  Amino acid sequence of Bs2FT
MKIVHISSGLGNQMFQYALYKKLSLIQDNVFLDTITSYQLYPNQHNGYELEKVFTIKPRHASKELTYNLSDLDNSVTSRIRRKLIGSKKSMYIEHKEFEYDPNLFYQENIYIKGYWQNYDYFKDIENELKNDFTFQRALDEKNNNLAIKINNENSISIHVRRGDYYLNRKNQEKFGDIANLEYYSKAISYIKERIDNPKFYIFSDNVEWVKQNLNSLEEAVYIDYNVGNDSYKDMQLMSLCKHNIIANSSFSWWGAFLNKNMEKIVIAPGKWINMKGVKKVNLFPKDWIIY

SEQ ID NO: 6 - DNA, 786 bp, Artificial Sequence
  Nucleotide sequence encoding Am2FT_2
atgaacatggaacggaaaaccggccttatgaataaaaaatatgtttccccgtgtttcctgcccggcatgcggctgggcaacatcatgttcacgctggcggccgcctgtgcccacgcccgtaccgtaggggtggagtgccgggtgccctgggcttacaatgacgcttccctgatgctgcgctcccggctcggcggctgggtgctcccttctacgccgtgcggcaccaatgaacctccatcctggcaggaaccttcctttgcctattgtccggttccctcccgcatccggacgggcgggcttcgcggctacttccagagcgcacggtattttgaagggcaggaagcgttcatccgggcgcttttcgcgcctctcaccgcggagaaggagcccggcgccgttggcattcacatccggcttggggactacaggcgcctccgtgacaagcaccgcattctggaccctggtttcctgcggagggccgcagggcatttatcatccgggaagaaccgtctggtgctgttcagcgatgagccggacgaggcggcggagatgcttgcgcgcgtgccggcattcggacgctttgcgctggaaatcgaccgcggcgctccgtgcgaatccctccgccgcatgacggcgatggaggaactcgtcatgtcgtgttcttccttttcctggtggggcgcgtggctgggaaatacccggaaggtcatcgttccgcgcgactggtttgtcggcggtgtggaagactaccgggatatttacctgccccattgggtaacactgtaa

SEQ ID NO: 7 - DNA, 876 bp, Artificial Sequence
  Nucleotide sequence encoding Bm2FT
atgaaaattgttcagatttcttctggtctgggtaaccagctgttccagtacgccctgtacaaacgtctgtctatgaacaacaacgatgtgttcctggatgtggagacgtcttatcaactgaacaaaaatcagcacaatggttacgaaattgaacgtattttttccatccagccatcccatgctaccaagggtatgatcgatgaactggccgatgtagacaaccgtctgatcaaccgcttacgtcgtaaactgtttggtccgaaaaactctatgtataccgaaaccaaagagttcagctacgattgtgaagttttcaccaaagatggtatctatatcaagggctactggcagaactataactattttaaagagattgaagacgatctgaaaaatgaactggtctttaaaaaagctctggatctgaaaaattcgcacctgatcaatcagatgaataaagaaattagcgtaagcatccacgtacgccgcggcgattattacctgaacaaggagtacgaaaacaaatttggcaacattgcggatcttgattattatctgaaagcgattaacttcatcaaaaaagaagtagacgatcccaaattttacgttttctccgacgatattaaatgggctaaagaaaatctgaacctgacggataacgtaacttatgttgaacacaacaaagggagcgactcttacaaagacatgcgtctgatgacctgctgtaaacataacatcatcgccaactctacattctcttggtggggcgcgtttcttaacgagaacaagaacaaaatcgtaatcgcgccgggcaaatggatcaacgttgaaggcgtcggtggcatcaacctgttccctgaaggttggatcgtttactga

SEQ ID NO: 8 - DNA, 900 bp, Artificial Sequence
  Nucleotide sequence encoding Bm2FT_2
atgggttgcataaaaagactattcttatatgaatacggaggacgatgttttttggtaattgttaaaataaaaggtggatttggtaaccaattgtttacatacgctagtgcttatgcaatatctcaagaactgcaacaaaacttaattatggataaggtaatatatgatctagattactttagaaaatttgaattaccttcattatcgttgaagtatgatcaaatgttaattagtaagtttgtacctaatactaaggttaaaactttaatttataaagttttaaggaggttaaaattaaaaggatttacagaggtacatgaaaaaaaggaattttcttttgatgaaaatatttacaatttgtcaggtgatatttatttagatggttattggcagaattatagatatttccataaatattataaagatctgtcggaaatgtttgtaccaagagaaactcctagaaaagaagtaactgattatatcacgtctttacggggagttaattctgttgctatgcatgttaggagaggagattataaaacttttaacggaggaaaatgtttgtctttagattattatattaaggctatggaatatttcaattcaaatgatgtacaattttatgtatttacagatgatattgatttttgtgagaaaaacctcccgaatagtgaaaatattaattatgtgtcaagaagcgagaaacttacagatattgaagaattctttattatgaaagaatgtaaaaattttataattgctaatagtagtttttcgtggtgggctgcttatttaagtgaacagaaagcagatagtttaattgtagcccctgttgttgacatgtggaaaagagatttttatccagatgagtgggtggcattgaatacacatttagaatag

SEQ ID NO: 9 - DNA, 864 bp, Artificial Sequence
  Nucleotide sequence encoding Bm2FT_3
atgataattgttcaaatcaagggcggattaggtaatcaacttttttcgtatgcttctgcttatggaattgcaagagagaatgaaacagaattaattattgatcgatatatatatgatacaagctactctttaagaaaatatatgttggattttttccctgagatcgatgaagcactacttctaaagtatatacctaaaaaaaataaaatttcacaaattatgtataaattgattagaaaatctaagttgaaatataagtacaaagctcaattatttttagaagaagaggaatttaagtttactagaattagtacccagaatgaaaatttgtatttaaatggttattggcaaagttatgtgtactttgataaatatcgtaatgacattattaaaaaattcacccctttagtaagctttaatcaagatggaaatcaacttcttaacgaaattaaaagttataattcagtggctatccatgtcaggagaggggattatattaattttaaaggtggaaagtgtttagatagttcttattatataaaggcaatgaagcatttatacaatttaaaaggaaaaaatttgtttttttatatttttacagatgatgtggaatattgtaaaagaatttttaaaaacgtagctaatgttaaatttataggtgaggaagcaaaattgagtgattttgaagagtttactttgatgactcattgtaaaaacctcataataggtaacagctcattttcttggtgggcagcttacttagcctcttgtaaagataaagctgtaatagctccagtggtagatatgtggactgaagatttctatctacctgaatggataaaaattaaagcggatttacaatag

SEQ ID NO: 10 - DNA, 876 bp, Artificial Sequence
  Nucleotide sequence encoding Bs2FT
atgaaaatagtacacataagtagcggtttaggaaatcaaatgtttcaatatgctctatataaaaaactgtccttaattcaagataatgtttttttggatacaattaccagttatcagttgtatcctaatcaacataatggatatgagttagagaaggtatttacaattaaaccaaggcatgcaagtaaagaattaacatacaatttatcagacttagataattcagtaacatctcgcattcgtaggaaattaattggaagtaaaaagagcatgtatatagaacataaagaatttgaatacgatcctaatttattttatcaagaaaatatatatataaaaggttactggcagaattatgattattttaaagatatagaaaatgaattaaagaatgattttacttttcaaagagctttagatgagaaaaataataatttagctattaaaattaacaatgagaattcaatatcaattcatgtaagacgtggtgattattacttaaacagaaagaatcaagagaagtttggagatatcgctaatttggaatactattcaaaggcaattagctatattaaagaaagaatagacaatccaaagttttatatcttttcagataatgttgagtgggtaaagcaaaatcttaattcgttagaggaagctgtatatatagattataacgtgggaaatgatagttacaaggatatgcaactaatgagtctttgtaaacataatattattgctaatagttcttttagttggtggggagcatttttgaataagaatatggagaaaatagttattgcacctgggaagtggattaatatgaaaggtgtaaaaaaagtcaatcttttcccaaaggattggataatttattaa

SEQ ID NO: 11 - DNA, 950 bp, Artificial Sequence
  p3610 promoter
caaatcttcctttcatctgctcatatatgatgctaatttacggatacaacataaaaaggcccatccgctcctagcataagctaggggcgaatggaccgcgttgccaccctaattagtacacataattgtgaactatctttattcatgtaacgttgaggtcaacgttcaagctttgcacttgaaagctccaaagtccattctgcaggtttcaatgtttgttctcaccagccacaaactctctgaaaatgaaaattctgcatactactctttttcacagctttaattatatagttattcgttattataacgcgaaaaagcaggaatttaaacatcttatcactaaaaagttttataagacaatttactgggatttttcagcggcaaaaaaagacaagaaccttttaattaaagcatttcttgatgaaaatttggtggaggatttggtaaaaatcttttatttaatatttctaatggctttgtaatactatcgtaatacctatactacaaaaaagattttagaagtctgacaagtaggcacaatccttataagataaggttttttcccccatgacaaaaaaataccattaaataatagtattgcaataaatttttaaaatatttataataggcgtaacaaacatattttttacaaaggtattacaatttcttaatttttcagaaaacacaaaatagacaatgttttgtttcaattagcgaattttgtaatgaatgagtcttctacatattaagcgcatacattggatttacagcatgtaaacaattgatgacagtttcatagagtagaagaataattttgcagtgaggtctttaatgctctactacatgaaaaaataactgattattttgtattgaaagaggattaagaaattagtgcatatcaaaaaaatatggttgccacacaaacaaaatttaatagggggtaacacgca

SEQ ID NO: 12 - DNA, 456 bp, Artificial Sequence
  p12455 promoter
agaagttctcctttccaaatagggcttataaaataattagcacttgagttgatagagtgctaattactcttcttatttaacatgtattggggtatttgtcaatatattaggagattcaccaaagagattaaaaattagactgaaaaaagcaaacttttaaaaaaaggttgaacgttctgaaagagtttgctagaatatacttaatttcaaagactatatgtgactggcgaaacgcggataaccgtgaggaagcatatagtgacgtagccgttcgcctgggcagaggtaagggattaatacatatctcttacctctttctgtttagggggagaggatatagaagttatcagacatgtaggctgaaaaaccagacttttaaaaaaattaaaaatgaagttcctttatccaaaggtaaaaacatgtaaaactacgatgataatcagaggagagtacaaa

SEQ ID NO: 13 - DNA, 398 bp, Artificial Sequence
  p24930 promoter
aaatctccactcctttacagaaaaaattccccatacctttctgtgtaaaacgtgaaaaacaaaattgagcctctgctcaactagacattaaatgatatacgaagcgcctcttttgaatatatatcttggaagaacattccttcaccccacgtaaagaaaatgcttacatttccatttgtttcaataacacacaaaatcaaaacatctgcatgtgtcattgctttgttacagccctataggtaaaacatacaattgtatgtaaaaagatgcggcctcaaaatatattataaacaattatctgacttttgtgaatcaaaagagagaagaaattttaaaaaaattattattatacaaaaatttctacgaaaaaagttcggttaatttcataaataaataag

SEQ ID NO: 14 - DNA, 390 bp, Artificial Sequence
  pTu promoter
aatgatgaaggttgaagttgttatccctgacgaatacttaggagatatcatgggtgacattacgtctcgtcgtggacgtgtagaaggtatggaagcacgcggtaacgctcaagttgtacgtgcattcgttccactttctgaaatgtttggttatgcaactgcattacgttcaaacactcaaggtcgcggaacatattctatgcacttcgatcactacgaagaagttcctaaatcaatttcagaagaaattattaaaaaaaataaaggtgaataattgattttcactctttattgaagtataactacttatgtacgctgtgaaagtggagttcattccctttcacggcctcataaaacataaactacatgaattttaaggaggattttcga

SEQ ID NO: 15 - DNA, 390 bp, Artificial Sequence
  pPDC promoter
aggagttaattcatgaaagtggcgatatcactattgtagcaggagctgattatgagttaaaagggaatcaaacatcttatgtaactgctaaacttccctattccaagcagctgtattccaaaacagtagacttgattcaaatgtcgcgcaatccaaactctaacaacattcacggtgaattcattggtctttggaaagtttccgcaaaaggcactgaggttgtaaaaaaagctttggaagaactggcgcaaagaaaagattttgctcagctcacgttttctgatttctttaattatgttaatctaattcacccggttgctgttaaatatacaatggggtcatggatagataccgaaacgtatacaaagattcaaaaagatggtgggaaaa

SEQ ID NO: 16 - DNA, 949 bp, Artificial Sequence
  p0706 promoter
caaatcttcctttcatctgcacatatatgatgctagtttaaggatacaacataaaaaggcccatccgctcctagcataagctaggggcgaatggaccgcgttgccaccctaattagcacacattattgtgaactatctttattcatgtaacgttgaggtcaacgttcaagctttgcacttgaaagctccaaagtccattctgcaggtttcaatgtttgttctcaccagccacaaactctctaaaaatgaaaattctgcatactactctttttcacagctttaattatatagttattcgttattataacgcgaaaaagcaggaatttaaacatcttatcgctaaaaagttttataagacaatttactggaatttttcagcgacaaaaaaagacaagaaccttttaattaaagcatttcttgatgaaaatttggtgtaggatttggtaaaaatcttttatttagtatttctaatagctctgtaatactattgtaatacctatactacaaaaaagattttagacgtctgacaagtaggcacgatccttataagataaggttttttccttcgccacaaaaaaatatcattagataatagtattgcaataaatttttaaaatatttataataggcgtaacaaacatattttttacaaaggtattacaatttcttaatttttcagaaaaaacaaaatagccaatgttttgtttcaattagcgaattttgtaatgaatgagccttctacatattaagcgcatacattggatttacagcatgtaaacaattgatgacagtttcatatagtagaagaataattttgctgtgagttctttaatgctctaccatacgaaaaaataactgattattttgtattgaaagaggattaagaaattggtgattattaaaaaatatggttgtcacacaaacaaaatttaatagggggtaacatgca

SEQ ID NO: 17 - protein, 587 aa, Artificial Sequence
  Amino acid sequence of lactose permease Lac12
MADHSSSSSSLQKKPINTIEHKDTLGNDRDHKEALNSDNDNTSGLKINGVPIEDAREEVLLPGYLSKQYYKLYGLCFITYLCATMQGYDGALMGSIYTEDAYLKYYHLDINSSSGTGLVFSIFNVGQICGAFFVPLMDWKGRKPAILIGCLGVVIGAIISSLTTTKSALIGGRWFVAFFATIANAAAPTYCAEVAPAHLRGKVAGLYNTLWSVGSIVAAFSTYGTNKNFPNSSKAFKIPLYLQMMFPGLVCIFGWLIPESPRWLVGVGREEEAREFIIKYHLNGDRTHPLLDMEMAEIIESFHGTDLSNPLEMLDVRSLFRTRSDRYRAMLVILMAWFGQFSGNNVCSYYLPTMLRNVGMKSVSLNVLMNGVYSIVTWISSICGAFFIDKIGRREGFLGSISGAALALTGLSICTARYEKTKKKSASNGALVFIYLFGGIFSFAFTPMQSMYSTEVSTNLTRSKAQLLNFVVSGVAQFVNQFATPKAMKNIKYWFYVFYVFFDIFEFIVIYFFFVETKGRSLEELEVVFEAPNPRKASVDQAFLAQVRATLVQRNDVRVANAQNLKEQEPLKSDADHVEKLSEAESV

SEQ ID NO: 18 - protein, 413 aa, Artificial Sequence
  Amino acid sequence of lactose permease LacY
MKSSKSLYWKLSAYFFFFFFTWSSSYSLFSIWLGQEIKLNGSATGLIFSVNAIFALCMQPLYGYISDRIGLKKHVLFFISCLLVFVGPFYIFVYGPLLQYNVVIGAIIGGLYLGVAFLAGIGAIETYIEKVSRKYKFEYGKSRMWGSLGWAAATFFAGQLFNINPHINFWVASVSAVILVAIIFSVKVEMSSYEMEKAESVTLRDVGSLFLLKEFWFFMIYVVGVTCVYGVYDQQFPIYYASLFPTESIGNQVFGYLNSFQVFLEAGMMFAAPFIVNKIGAKNSLILAGFLMGFRIIGSGLVVGPIGISSMKLIHALELPIMLIAIFKYLAANFDTRLSSILYLVGFQFASQIGASVLSPIVGGLYDSVGFSRTYLIMGGMVLVFNVISMFTLLNSKKHRFIRKDVQENTQII

SEQ ID NO: 19 - DNA, 1764 bp, Artificial Sequence
  Nucleotide sequence encoding lactose permease Lac12
atggctgatcactcttcttcttcttcttctttacaaaaaaaaccaattaacacaattgaacacaaagatacattaggtaacgatcgtgatcacaaagaagctttaaactctgataacgataacacatctggtttaaaaattaacggtgtaccaattgaagatgctcgtgaagaagtattattaccaggttacttatctaaacaatactacaaattatacggtttatgtttcattacatacttatgtgctacaatgcaaggttacgatggtgctttaatgggttctatttacacagaagatgcttacttaaaatactaccacttagatattaactcttcttctggtacaggtttagtattctctattttcaacgtaggtcaaatttgtggtgctttcttcgtaccattaatggattggaaaggtcgtaaaccagctattttaattggttgtttaggtgtagtaattggtgctattatttcttctttaacaacaacaaaatctgctttaattggtggtcgttggttcgtagctttcttcgctacaattgctaacgctgctgctccaacatactgtgctgaagtagctccagctcacttacgtggtaaagtagctggtttatacaacacattatggtctgtaggttctattgtagctgctttctctacatacggtacaaacaaaaacttcccaaactcttctaaagctttcaaaattccattatacttacaaatgatgttcccaggtttagtatgtattttcggttggttaattccagaatctccacgttggttagtaggtgtaggtcgtgaagaagaagctcgtgaattcattattaaataccacttaaacggtgatcgtacacacccattattagatatggaaatggctgaaattattgaatctttccacggtacagatttatctaacccattagaaatgttagatgtacgttctttattccgtacacgttctgatcgttaccgtgctatgttagtaattttaatggcttggttcggtcaattctctggtaacaacgtatgttcttactacttaccaacaatgttacgtaacgtaggtatgaaatctgtatctttaaacgtattaatgaacggtgtatactctattgtaacatggatttcttctatttgtggtgctttcttcattgataaaattggtcgtcgtgaaggtttcttaggttctatttctggtgctgctttagctttaacaggtttatctatttgtacagctcgttacgaaaaaacaaaaaaaaaatctgcttctaacggtgctttagtattcatttacttattcggtggtattttctctttcgctttcacaccaatgcaatctatgtactctacagaagtatctacaaacttaacacgttctaaagctcaattattaaacttcgtagtatctggtgtagctcaattcgtaaaccaattcgctacaccaaaagctatgaaaaacattaaatactggttctacgtattctacgtattcttcgatattttcgaattcattgtaatttacttcttcttcgtagaaacaaaaggtcgttctttagaagaattagaagtagtattcgaagctccaaacccacgtaaagcttctgtagatcaagctttcttagctcaagtacgtgctacattagtacaacgtaacgatgtacgtgtagctaacgctcaaaacttaaaagaacaagaaccattaaaatctgatgctgatcacgtagaaaaattatctgaagctgaatctgtataa

SEQ ID NO: 20 - DNA, 1242 bp, Artificial Sequence
  Nucleotide sequence encoding lactose permease LacY
atgaaaagttcaaaaagtttatattggaagctgagtgcatattttttcttcttcttttttacgtggtcgtccagctactctttattttctatctggttagggcaagagattaagttgaacggatcagcaacaggcttaatcttttctgtgaacgctatctttgctttgtgtatgcagcctttgtacggatatatatctgacaggataggtttaaagaaacacgttttattttttattagctgtcttttagtgtttgtaggaccattttatatttttgtttatggacctttgcttcaatacaatgtggtgataggggctattattggaggcttatatttaggagtagcgtttttggcgggcatcggagcgattgaaacatacatagagaaagtcagccgaaaatataaatttgagtatggaaaatctagaatgtgggggtcattaggctgggctgcagctacgttttttgcaggacaattatttaatattaatcctcacattaatttttgggtggcatctgtttcagcggttatcctagtcgctattattttttctgtaaaagtagaaatgagcagttatgaaatggaaaaagctgaatccgtcacgctaagagatgtaggtagtttatttttattgaaggaattttggttttttatgatttatgttgttggtgttacatgcgtatatggggtatacgatcagcaatttcctatctattatgcatctttgtttcctactgaatcgataggtaaccaagtatttggctacttaaattcgtttcaagtatttttagaagctggaatgatgttcgcagcaccgtttattgtaaataagatcggtgcaaaaaatagtttaattttagcaggatttctaatgggatttcgtattattgggtcagggcttgttgttggtccaatcggaatatcttcaatgaaactcattcatgcattagaacttcctattatgctcattgccatctttaaatatttggcagctaactttgacacgcgcctatcttccatcctttatttggttggattccaatttgcttcgcaaataggtgcttcagttctttcacccatagtgggaggattatatgatagcgtaggtttttcccgtacctatttaattatgggaggtatggttttggtatttaacgttatttcgatgtttacactactaaactctaaaaaacatagatttataagaaaagatgtacaagaaaacacgcagattatatag

SEQ ID NO: 21 - DNA, 11 bp, Artificial Sequence
  RBS
aaagggggaaa

SEQ ID NO: 22 - DNA, 11 bp, Artificial Sequence
  RBS
gaaggaggtga

SEQ ID NO: 23 - protein, 462 aa, Artificial Sequence
  Amino acid sequence of GTP-mannose-1-phosphate guanylyltransferase
MKLVLLSGGSGKRLWPLSNDTRSKQFLKVLEGRDGQKESMVQRVWSQIEAVGLNESTVIATSKLQRDMITGQVGTDIPLIIEPERRDTFPAIALAASYLHSEEQASEDEIVVVLPVDPYVEDGFFERVKDLESVLRDSKADLALMGVTPTYPSSKYGYIVPEGKVQGDSYFTVDCFTEKPSEEAAVGLINQRALWNCGVFAFRLGYLLQILQEKKLPLQFETLHKEYATLPKISFDYEVVEKASHIVALPYDGYWKDLGTWNTLTEEMATSQIGKGVLTDDSANTHLVNELDIPVTVLGVKDVVVAASPDGILVADKASSPKIKEIIGDWNYPPMYEERLWGWSRVLDYAKYDEETEMVTKRIHISKGKNSTYHYHNLRDEVWTIVRGEGELALDDYIRRVKAGDIIHLPAGKKHGIHALTDLEFIEVQTGKVISNEDSIRLIYDWNDVIKQFQSSRPQVIL

SEQ ID NO: 24 - protein, 359 aa, Artificial Sequence
  Amino acid sequence of phosphomannomurase
LKTIAYYISDYGYGHATRSTAIIRQLLKQNEEIEIIICHSFAIEFLRQSFRYERRVRFREILTDVGYVLKENSLEPDADLLNRQVASYVSSFHTKLMYEKHFMKVANVSFVISDISPLGIAGAYLLKLPSLGISNFTWFTAYEGLIGELSLEFLEKRYKQMTYQFSLACSDEPHWGIKENQSFGFYSREINDSEVQRIRKEIDPEGESYIIYFGLGMKVDIGTLSDLPIWQSPNCKFIVSSNVDVTHPNVYKIPQDETETQHYVAAADLGLTKAGWGTISEAVCAGVPLLITNRSSMKEDRHTIDYLVRHQLCDLIEWKELEGLVVTPSLIETCRRQQINRYKNEAMHIAEEINKKINS

SEQ ID NO: 25 - protein, 313 aa, Artificial Sequence
  Amino acid sequence of GDP-L-fucose synthase
MNKNSKIYVAGHRGLVGSAIVRKLQEKGYSNLVYRTSAELDLRDKPTVDAFFAEEKPEFVFLAAAKVGGIVANNEYPAEFIHDNLLIQSNIIDAAYRNDVEKLLFLGSTCIYPKLAPQPLKEEYLLTGELEPTNEPYAIAKIAGIKMCESYNRQYGTKYISAMPTNLYGPNDNFDLHTSHVLPALLRKFHEAKESNAPFVEMWGTGTPKREFLYSDDLADACVFLMNTYEGNEIVNIGVGEDITIKELGEKVKAVVGYEGNIQFDTSKPDGTPRKLVDVTKLNSLGWKAETALEDGLQKAYQWFLDNELAAAK

SEQ ID NO: 26 - protein, 359 aa, Artificial Sequence
  Amino acid sequence of GDP-D-mannose-4,6-dehydratase
MKTALITGVTGQDGSYLAELLLEKGYEVHGLIRRSSSYNQERLEDLLTEEAASALLNNSNFHLHYGDVTDALNVTRIIGDIQPDEIYNLAAQSHVRVSFDMPGYTLDVDAKGTLNILEAVRILGLTDKTRVYQASTSELYGKVQEVPQKETTPFYPRSPYGVAKIYGFWITKNYRESYSMFAVNGILFNHESERRGETFVTRKITLAASRIAQGKQQKLTLGNLDSLRDWGYAKDYVECMWLILQHDKPEDFVIATGEMHSVREFVQLAFKHTGIEIEWSGEGLEEKGTNKATGEVIVEIDPKFFRPAEVDQLLGDPTKAKTLLKWNPTKTSFEELVRIMVEADMKKVESEEKIKVMFD

SEQ ID NO: 27 - DNA, 1389 bp, Artificial Sequence
  Nucleotide sequence encoding GTP-mannose-1-phosphate guanylyltransferase
atgaaacttgtattgttatcgggtggatctggtaagcgtctatggccgttatcaaatgatacgcgttcgaagcagtttttaaaggtattagaaggacgagatggacagaaagagtcaatggttcagcgcgtctggagtcaaattgaagcggttgggttaaatgagtcaacggttattgcgacgtctaagcttcagcgtgatatgattacaggtcaggttggcaccgatattccgttgattattgaacctgagcgccgcgatacgtttccagcgattgctttagctgcttcatatcttcattccgaagagcaagcatctgaagatgaaatcgttgtggtgttgccagttgacccttatgtggaagacggattttttgaacgggtaaaagatttagaaagtgtgcttcgtgattcaaaagcggatttagcgttaatgggtgttacacctacgtatccttcatctaagtacgggtacatcgtgccggaaggaaaggtacaaggggacagttattttacagtggattgttttacagaaaagccgagtgaagaagcagctgttggattaattaatcagcgtgcgctttggaactgcggcgtttttgcgtttcgtttaggttatttgcttcaaattttacaagagaaaaaacttccacttcaatttgaaacgctacataaagaatatgcaacattgcctaaaattagttttgactatgaagtggtggaaaaggcaagtcatattgtcgcgcttccgtatgatgggtactggaaagatcttggtacatggaatacgttaacggaagaaatggcgacatctcaaattggaaaaggtgtattaacggacgactcagctaatacgcatttagtgaatgaattagatattccggttacggtattaggcgtaaaagatgtagttgttgccgctagtccagatgggatcttagttgcggataaagcatctagtcctaagattaaagaaattattggcgactggaactaccctccaatgtatgaagaacgtctttggggctggtcacgcgtgttagattatgcaaagtatgatgaagaaactgaaatggtgacaaaacgtattcatatttcaaaaggaaagaactcgacgtatcactatcataatttacgtgatgaagtatggacgattgtacgtggagaaggagagcttgcgcttgatgactacattcgccgcgtaaaagcaggggatattattcacttgccggctggcaaaaagcacggaattcatgcgttaaccgaccttgaatttattgaagtacaaacgggaaaagtgatttcaaatgaagatagtattcgccttatttatgactggaatgatgtgatcaagcaattccaatcatcaagaccgcaggtgattttataa

SEQ ID NO: 28 - DNA, 1080 bp, Artificial Sequence
  Nucleotide sequence encoding phosphomannomurase
ttgaaaacaattgcctattacatttcagactacggatatggccacgcgactagaagcacggccattattcgtcaattattaaagcaaaatgaagaaatagaaattattatttgtcattcatttgcgattgagtttctcagacaatcttttagatatgaacgtcgtgtgaggtttcgagagattttaacggatgtcggctacgtgctaaaagaaaattcactagaaccagacgctgatttgttgaatcgtcaagttgcttcttatgtatcaagctttcatacgaagcttatgtatgagaagcactttatgaaagtagccaacgtttcattcgtgatttcggatatttctccgttagggatcgcaggtgcctatctattaaaattgccttctttaggaatatcaaatttcacttggtttacagcatacgaagggttaattggagagctatcgctggaatttttagaaaaacgttataagcagatgacgtatcagttttcgctagcatgtagtgatgagccacattggggtatcaaagaaaatcaaagctttggtttttattcaagagaaataaacgattctgaagtacagcgtattcgtaaagagattgatcctgaaggtgagagttacatcatctacttcggtctgggtatgaaagtagatattggaacgttgtcggacttgcctatttggcaaagtccaaactgcaagtttatcgtttcatcgaatgttgatgttactcatcccaatgtttataaaattcctcaagatgaaacagaaacgcagcactatgtagcagcagctgatcttggtttaacaaaagcaggctggggcacgattagtgaagcggtttgcgctggtgtgccgctgttgattacaaatcgcagcagcatgaaagaagatcgtcatacgattgattatttagttcgtcatcagctatgcgacttaatagagtggaaagagttagaaggtttagtagtaactccttcgcttattgagacatgcaggcggcagcaaatcaatcgctataaaaatgaagcgatgcatatcgccgaagaaatcaataaaaaaataaacagttag

SEQ ID NO: 29 - DNA, 942 bp, Artificial Sequence
  Nucleotide sequence encoding GDP-L-fucose synthase
atgaacaaaaattcgaaaatttacgtagctggtcatagaggtctcgtcggttcagctatcgtacgaaaactacaagaaaaaggctatagcaatctagtgtatcgcacaagcgctgagctagatttaagagacaagccgacagtagacgcattctttgctgaagaaaagccagaatttgttttcttagcagccgctaaagtaggtggtattgtggcaaacaatgaatatccagcggaatttattcacgataacttattgattcaatcaaatattattgatgcagcatatcgcaatgatgtagagaaactattattcctaggaagtacatgtatttatccaaaattagcgcctcagccattaaaagaagaatacttactaacaggtgagctggagccaacaaacgaaccgtatgcaattgctaaaattgctggaatcaaaatgtgtgaatcctataaccgtcagtacggaacaaaatatatctcggcaatgcctactaacctttacggtccaaacgacaattttgaccttcatacatcacacgttcttcctgcactgcttcgtaagttccatgaagcgaaagaaagcaatgcgccgtttgttgaaatgtggggaacaggcacaccaaaacgtgaatttctatattcagatgacctagcagatgcgtgcgtattcttaatgaatacatatgaaggcaatgaaatcgttaatatcggtgtgggagaagatattacgattaaagaacttggcgaaaaagtaaaagcagttgttggttatgaaggaaatattcagtttgatacgtcaaaaccagacggaacgcctcgtaaactagtagacgtaacaaaattgaacagtcttggctggaaagcagaaacagctttagaagacggtcttcaaaaagcgtatcagtggtttttagataacgaactagctgcagcaaaataa

SEQ ID NO: 30 - DNA, 1080 bp, Artificial Sequence
  Nucleotide sequence encoding GDP-D-mannose-4,6-dehydratase
atgaaaacagcattaattacaggtgtaacaggacaagatggatcatacttagcagaacttttactagaaaaaggctatgaagtgcacggactaattcgccgcagctcttcttataaccaagagcgtctagaagatcttttaacagaagaagcagcgagcgcattattaaacaactcaaacttccaccttcactatggtgacgtaacagatgcattaaatgttactcgtattattggtgacattcagccagatgaaatttacaatctagctgcacagtcacatgtacgtgtgtcttttgatatgcctggatatacattagatgttgatgcaaaaggtacgttaaacattcttgaagctgtacgtattttagggttaacagataaaacacgtgtgtaccaagcttctacatctgaactgtacggaaaagttcaagaagtaccacaaaaggaaacaacacctttctaccctcgttctccatatggcgtagcgaaaatttacggcttttggattacaaagaactaccgtgaatcttatagcatgtttgcagtaaacggtattttatttaaccatgaatcagagcgccgcggcgaaacgttcgtaacacgtaaaattacgcttgctgcttcacgtatcgcgcaaggcaagcagcaaaaattaacgcttggaaacttagactctttacgtgactggggttacgcaaaagactatgtagaatgcatgtggttaattcttcaacacgataaacctgaagattttgttattgcgactggtgaaatgcactcagtacgtgaatttgtacagcttgcattcaaacatacaggcattgaaattgagtggagcggtgaaggtctagaagaaaaaggaacaaataaagcaacgggtgaagtgatcgtagaaatcgatcctaagttcttccgtcctgcagaagtggatcaattgttaggtgatccaactaaagccaagactttattaaagtggaaccccactaagacttcgtttgaagaattagttcgcattatggtggaagcggacatgaagaaggttgaaagcgaagagaagattaaggtgatgtttgattaa

SEQ ID NO: 31 - DNA, 9 bp, Artificial Sequence
  RBS
aaggaggtg